European Patent Specification EP 3 355 915 B1, published November 1, 2023. Title: Canine Parvovirus (CPV) Virus-like Particle (VLP) Vaccines and uses thereof. Applicant: Merial, Inc. David, Frederic Hannas-Djebbara , Zahia Poulet, Herve Minke, Jules. The sequence listing filed with the application follows.

SEQUENCE LISTING (12 sequences)

SEQ ID NO: 1 - protein, 584 aa, Artificial Sequence
  VP2 of Canine parvovirus - GenBank BAD34656.1
MSDGAVQPDGGQPAVRNERATGSGNGSGGGGGGGSGGVGISTGTFNNQTEFKFLENGWVEITANSSRLVHLNMPESENYRRVVVNNLDKTAVNGNMALDDTHAQIVTPWSLVDANAWGVWFNPGDWQLIVNTMSELHLVSFEQEIFNVVLKTVSESATQPPTKVYNNDLTASLMVALDSNNTMPFTPAAMRSETLGFYPWKPTIPTPWRYYFQWDRTLIPSHTGTSGTPTNIYHGTDPDDVQFYTIENSVPVHLLRTGDEFATGTFFFDCKPCRLTHTWQTNRALGLPPFLNSLPQAEGGTNFGYIGVQQDKRRGVTQMGNTNYITEATIMRPAEVGYSAPYYSFEASTQGPFKTPIAAGRGGAQTDENQAADGDPRYAFGRQHGQKTTTTGETPERFTYIAHQDTGRYPEGDWIQNINFNLPVTEDNVLLPTDPIGGKTGINYTNIFNTYGPLTALNNVPPVYPNGQIWDKEFDTDLKPRLHVNAPFVCQNNCPGQLFVKVAPNLTNEYDPDASANMSRIVTYSDFWWKGKLVFKAKLRASHTWNPIQQMSINVDNQFNYVPSNIGGMKIVYEKSQLAPRKLY

SEQ ID NO: 2 - DNA, 9632 bp, Artificial Sequence
  pVL1393 - 9632 bp baculovirus transfer vector from Invitrogen
aagctttactcgtaaagcgagttgaaggatcatatttagttgcgtttatgagataagattgaaagcacgtgtaaaatgtttcccgcgcgttggcacaactatttacaatgcggccaagttataaaagattctaatctgatatgttttaaaacacctttgcggcccgagttgtttgcgtacgtgactagcgaagaagatgtgtggaccgcagaacagatagtaaaacaaaaccctagtattggagcaataatcgatttaaccaacacgtctaaatattatgatggtgtgcattttttgcgggcgggcctgttatacaaaaaaattcaagtacctggccagactttgccgcctgaaagcatagttcaagaatttattgacacggtaaaagaatttacagaaaagtgtcccggcatgttggtgggcgtgcactgcacacacggtattaatcgcaccggttacatggtgtgcagatatttaatgcacaccctgggtattgcgccgcaggaagccatagatagattcgaaaaagccagaggtcacaaaattgaaagacaaaattacgttcaagatttattaatttaattaatattatttgcattctttaacaaatactttatcctattttcaaattgttgcgcttcttccagcgaaccaaaactatgcttcgcttgctccgtttagcttgtagccgatcagtggcgttgttccaatcgacggtaggattaggccggatattctccaccacaatgttggcaacgttgatgttacgtttatgcttttggttttccacgtacgtcttttggccggtaatagccgtaaacgtagtgccgtcgcgcgtcacgcacaacaccggatgtttgcgcttgtccgcggggtattgaaccgcgcgatccgacaaatccaccactttggcaactaaatcggtgacctgcgcgtcttttttctgcattatttcgtctttcttttgcatggtttcctggaagccggtgtacatgcggtttagatcagtcatgacgcgcgtgacctgcaaatctttggcctcgatctgcttgtccttgatggcaacgatgcgttcaataaactcttgttttttaacaagttcctcggttttttgcgccaccaccgcttgcagcgcgtttgtgtgctcggtgaatgtcgcaatcagcttagtcaccaactgtttgctctcctcctcccgttgtttgatcgcgggatcgtacttgccggtgcagagcacttgaggaattacttcttctaaaagccattcttgtaattctatggcgtaaggcaatttggacttcataatcagctgaatcacgccggatttagtaatgagcactgtatgcggctgcaaatacagcgggtcgccccttttcacgacgctgttagaggtagggcccccattttggatggtctgctcaaataacgatttgtatttattgtctacatgaacacgtatagctttatcacaaactgtatattttaaactgttagcgacgtccttggccacgaaccggacctgttggtcgcgctctagcacgtaccgcaggttgaacgtatcttctccaaatttaaattctccaattttaacgcgagccattttgatacacgtgtgtcgattttgcaacaactattgttttttaacgcaaactaaacttattgtggtaagcaataattaaatatgggggaacatgcgccgctacaacactcgtcgttatgaacgcagacggcgccggtctcggcgcaagcggctaaaacgtgttgcgcgttcaacgcggcaaacatcgcaaaagccaatagtacagttttgatttgcatattaacggcgattttttaaattatcttatttaataaatagttatgacgcctacaactccccgcccgcgttgactcgctgcacctcgagcagttcgttgacgccttcctccgtgtggccgaacacgtcgagcgggtggtcgatgaccagcggcgtgccgcacgcgacgcacaagtatctgtacaccgaatgatcgtcgggcgaaggcacgtcggcctccaagtggcaatattggcaaattcgaaaatatatacagttgggttgtttgcgcatatctatcgtggcgttgggcatgtacgtccgaacgttgatttgcatgcaagccgaaattaaatcattgcgattagtgcgattaaaacgttgtacatcctcgcttttaatcatgccgtcgattaaatcgcgcaatcgagtcaagtgatcaaagtgtggaataatgttttctttgtattcccgagtcaagcgcagcgcgtattttaacaaactagccatcttgtaagttagtttcatttaatgcaactttatccaataatatattatgtatcgcacgtcaagaattaacaatgcgcccgttgtcgcatctcaacacgactatgatagagatcaaataaagcgcgaattaaatagcttgcgacgcaacgtgcacgatctgtgcacgcgttccggcacgagctttgattgtaataagtttttacgaagcgatgacatgacccccgtagtgacaacgatcacgcccaaaagaactgccgactacaaaattaccgagtatgtcggtgacgttaaaactattaagccatccaatcgaccgttagtcgaatcaggaccgctggtgcgagaagccgcgaagtatggcgaatgcatcgtataacgtgtggagtccgctcattagagcgtcatgtttagacaagaaagctacatatttaattgatcccgatgattttattgataaattgaccctaactccatacacggtattctacaatggcggggttttggtcaaaatttccggactgcgattgtacatgctgttaacggctccgcccactattaatgaaattaaaaattccaattttaaaaaacgcagcaagagaaacatttgtatgaaagaatgcgtagaaggaaagaaaaatgtcgtcgacatgctgaacaacaagattaatatgcctccgtgtataaaaaaaatattgaacgatttgaaagaaaacaatgtaccgcgcggcggtatgtacaggaagaggtttatactaaactgttacattgcaaacgtggtttcgtgtgccaagtgtgaaaaccgatgtttaatcaaggctctgacgcatttctacaaccacgactccaagtgtgtgggtgaagtcatgcatcttttaatcaaatcccaagatgtgtataaaccaccaaactgccaaaaaatgaaaactgtcgacaagctctgtccgtttgctggcaactgcaagggtctcaatcctatttgtaattattgaataataaaacaattataaatgctaaatttgttttttattaacgatacaaaccaaacgcaacaagaacatttgtagtattatctataattgaaaacgcgtagttataatcgctgaggtaatatttaaaatcattttcaaatgattcacagttaatttgcgacaatataattttattttcacataaactagacgccttgtcgtcttcttcttcgtattccttctctttttcatttttctcctcataaaaattaacatagttattatcgtatccatatatgtatctatcgtatagagtaaattttttgttgtcataaatatatatgtcttttttaatggggtgtatagtaccgctgcgcatagtttttctgtaatttacaacagtgctattttctggtagttcttcggagtgtgttgctttaattattaaatttatataatcaatgaatttgggatcgtcggttttgtacaatatgttgccggcatagtacgcagcttcttctagttcaattacaccattttttagcagcaccggattaacataactttccaaaatgttgtacgaaccgttaaacaaaaacagttcacctcccttttctatactattgtctgcgagcagttgtttgttgttaaaaataacagccattgtaatgagacgcacaaactaatatcacaaactggaaatgtctatcaatatatagttgctgatatcatggagataattaaaatgataaccatctcgcaaataaataagtattttactgttttcgtaacagttttgtaataaaaaaacctataaatattccggattattcataccgtcccaccatcgggcgcggatcccgggtaccttctagaattccggagcggccgctgcagatctgatcctttcctgggacccggcaagaaccaaaaactcactctcttcaaggaaatccgtaatgttaaacccgacacgatgaagcttgtcgttggatggaaaggaaaagagttctacagggaaacttggacccgcttcatggaagacagcttccccattgttaacgaccaagaagtgatggatgttttccttgttgtcaacatgcgtcccactagacccaaccgttgttacaaattcctggcccaacacgctctgcgttgcgaccccgactatgtacctcatgacgtgattaggatcgtcgagccttcatgggtgggcagcaacaacgagtaccgcatcagcctggctaagaagggcggcggctgcccaataatgaaccttcactctgagtacaccaactcgttcgaacagttcatcgatcgtgtcatctgggagaacttctacaagcccatcgtttacatcggtaccgactctgctgaagaggaggaaattctccttgaagtttccctggtgttcaaagtaaaggagtttgcaccagacgcacctctgttcactggtccggcgtattaaaacacgatacattgttattagtacatttattaagcgctagattctgtgcgttgttgatttacagacaattgttgtacgtattttaataattcattaaatttataatctttagggtggtatgttagagcgaaaatcaaatgattttcagcgtctttatatctgaatttaaatattaaatcctcaatagatttgtaaaataggtttcgattagtttcaaacaagggttgtttttccgaaccgatggctggactatctaatggattttcgctcaacgccacaaaacttgccaaatcttgtagcagcaatctagctttgtcgatattcgtttgtgttttgttttgtaataaaggttcgacgtcgttcaaaatattatgcgcttttgtatttctttcatcactgtcgttagtgtacaattgactcgacgtaaacacgttaaataaagcttggacatatttaacatcgggcgtgttagctttattaggccgattatcgtcgtcgtcccaaccctcgtcgttagaagttgcttccgaagacgattttgccatagccacacgacgcctattaattgtgtcggctaacacgtccgcgatcaaatttgtagttgagctttttggaattatttctgattgcgggcgtttttgggcgggtttcaatctaactgtgcccgattttaattcagacaacacgttagaaagcgatggtgcaggcggtggtaacatttcagacggcaaatctactaatggcggcggtggtggagctgatgataaatctaccatcggtggaggcgcaggcggggctggcggcggaggcggaggcggaggtggtggcggtgatgcagacggcggtttaggctcaaatgtctctttaggcaacacagtcggcacctcaactattgtactggtttcgggcgccgtttttggtttgaccggtctgagacgagtgcgatttttttcgtttctaatagcttccaacaattgttgtctgtcgtctaaaggtgcagcgggttgaggttccgtcggcattggtggagcgggcggcaattcagacatcgatggtggtggtggtggtggaggcgctggaatgttaggcacgggagaaggtggtggcggcggtgccgccggtataatttgttctggtttagtttgttcgcgcacgattgtgggcaccggcgcaggcgccgctggctgcacaacggaaggtcgtctgcttcgaggcagcgcttggggtggtggcaattcaatattataattggaatacaaatcgtaaaaatctgctataagcattgtaatttcgctatcgtttaccgtgccgatatttaacaaccgctcaatgtaagcaattgtattgtaaagagattgtctcaagctcgccgcacgccgataacaagccttttcatttttactacagcattgtagtggcgagacacttcgctgtcgtcgacgtacatgtatgctttgttgtcaaaaacgtcgttggcaagctttaaaatatttaaaagaacatctctgttcagcaccactgtgttgtcgtaaatgttgtttttgataatttgcgcttccgcagtatcgacacgttcaaaaaattgatgcgcatcaattttgttgttcctattattgaataaataagattgtacagattcatatctacgattcgtcatggccaccacaaatgctacgctgcaaacgctggtacaattttacgaaaactgcaaaaacgtcaaaactcggtataaaataatcaacgggcgctttggcaaaatatctattttatcgcacaagcccactagcaaattgtatttgcagaaaacaatttcggcgcacaattttaacgctgacgaaataaaagttcaccagttaatgagcgaccacccaaattttataaaaatctattttaatcacggttccatcaacaaccaagtgatcgtgatggactacattgactgtcccgatttatttgaaacactacaaattaaaggcgagctttcgtaccaacttgttagcaatattattagacagctgtgtgaagcgctcaacgatttgcacaagcacaatttcatacacaacgacataaaactcgaaaatgtcttatatttcgaagcacttgatcgcgtgtatgtttgcgattacggattgtgcaaacacgaaaactcacttagcgtgcacgacggcacgttggagtattttagtccggaaaaaattcgacacacaactatgcacgtttcgtttgactggtacgcggcgtgttaacatacaagttgctaacgtaatcatggtcatagctgtttcctgtgtgaaattgttatccgctcacaattccacacaacatacgagccggaagcataaagtgtaaagcctggggtgcctaatgagtgagctaactcacattaattgcgttgcgctcactgcccgctttccagtcgggaaacctgtcgtgccagctgcattaatgaatcggccaacgcgcggggagaggcggtttgcgtattgggcgctcttccgcttcctcgctcactgactcgctgcgctcggtcgttcggctgcggcgagcggtatcagctcactcaaaggcggtaatacggttatccacagaatcaggggataacgcaggaaagaacatgtgagcaaaaggccagcaaaaggccaggaaccgtaaaaaggccgcgttgctggcgtttttccataggctccgcccccctgacgagcatcacaaaaatcgacgctcaagtcagaggtggcgaaacccgacaggactataaagataccaggcgtttccccctggaagctccctcgtgcgctctcctgttccgaccctgccgcttaccggatacctgtccgcctttctcccttcgggaagcgtggcgctttctcatagctcacgctgtaggtatctcagttcggtgtaggtcgttcgctccaagctgggctgtgtgcacgaaccccccgttcagcccgaccgctgcgccttatccggtaactatcgtcttgagtccaacccggtaagacacgacttatcgccactggcagcagccactggtaacaggattagcagagcgaggtatgtaggcggtgctacagagttcttgaagtggtggcctaactacggctacactagaaggacagtatttggtatctgcgctctgctgaagccagttaccttcggaaaaagagttggtagctcttgatccggcaaacaaaccaccgctggtagcggtggtttttttgtttgcaagcagcagattacgcgcagaaaaaaaggatctcaagaagatcctttgatcttttctacggggtctgacgctcagtggaacgaaaactcacgttaagggattttggtcatgagattatcaaaaaggatcttcacctagatccttttaaattaaaaatgaagttttaaatcaatctaaagtatatatgagtaaacttggtctgacagttaccaatgcttaatcagtgaggcacctatctcagcgatctgtctatttcgttcatccatagttgcctgactccccgtcgtgtagataactacgatacgggagggcttaccatctggccccagtgctgcaatgataccgcgagacccacgctcaccggctccagatttatcagcaataaaccagccagccggaagggccgagcgcagaagtggtcctgcaactttatccgcctccatccagtctattaattgttgccgggaagctagagtaagtagttcgccagttaatagtttgcgcaacgttgttgccattgctacaggcatcgtggtgtcacgctcgtcgtttggtatggcttcattcagctccggttcccaacgatcaaggcgagttacatgatcccccatgttgtgcaaaaaagcggttagctccttcggtcctccgatcgttgtcagaagtaagttggccgcagtgttatcactcatggttatggcagcactgcataattctcttactgtcatgccatccgtaagatgcttttctgtgactggtgagtactcaaccaagtcattctgagaatagtgtatgcggcgaccgagttgctcttgcccggcgtcaatacgggataataccgcgccacatagcagaactttaaaagtgctcatcattggaaaacgttcttcggggcgaaaactctcaaggatcttaccgctgttgagatccagttcgatgtaacccactcgtgcacccaactgatcttcagcatcttttactttcaccagcgtttctgggtgagcaaaaacaggaaggcaaaatgccgcaaaaaagggaataagggcgacacggaaatgttgaatactcatactcttcctttttcaatattattgaagcatttatcagggttattgtctcatgagcggatacatatttgaatgtatttagaaaaataaacaaataggggttccgcgcacatttccccgaaaagtgccacctgacgtctaagaaaccattattatcatgacattaacctataaaaataggcgtatcacgaggccctttcgtctcgcgcgtttcggtgatgacggtgaaaacctctgacacatgcagctcccggagacggtcacagcttgtctgtaagcggatgccgggagcagacaagcccgtcagggcgcgtcagcgggtgttggcgggtgtcggggctggcttaactatgcggcatcagagcagattgtactgagagtgcaccatatgcggtgtgaaataccgcacagatgcgtaaggagaaaataccgcatcaggcgccattcgccattcaggctgcgcaactgttgggaagggcgatcggtgcgggcctcttcgctattacgccagctggcgaaagggggatgtgctgcaaggcgattaagttgggtaacgccagggttttcccagtcacgacgttgtaaaacgacggccagtgcc

SEQ ID NO: 3 - protein, 584 aa, Artificial Sequence; identical to SEQ ID NO: 1
  CPV Souriou (serotype 2c)

SEQ ID NO: 4 - protein, 584 aa, Artificial Sequence; identical to SEQ ID NO: 1
  Non-Truncated CPV VP2 in pMEB072

SEQ ID NO: 5 - DNA, 1752 bp, Artificial Sequence
  pMEB072 Codon-optimized nucleic acid encoding CPV VP2 (SEQ ID NO:4)
atgtccgacggtgctgtgcagcccgacggtggccagcccgctgtgcgtaacgagcgtgctaccggttccggtaacggttcaggcggaggtggaggtggtggttccggcggtgtgggcatctccaccggcaccttcaacaaccagaccgagttcaagttcctcgagaacggttgggtggagatcaccgctaactcctcccgtctggtgcacctgaacatgcccgagtccgagaactaccgtcgtgtggtggtgaacaacctggacaagaccgctgtgaacggtaacatggctctggacgacacccacgctcagatcgtgaccccctggtccctggtggacgctaacgcttggggcgtgtggttcaaccccggtgactggcagctgatcgtgaacaccatgtccgagctgcacctggtgtccttcgagcaagagatcttcaacgtcgtcctcaagaccgtgtccgagtccgctacccagccccccaccaaggtgtacaacaacgacctgaccgcttccctgatggtcgctctggactccaacaacaccatgcccttcacccccgctgctatgcgttccgagaccctgggcttctacccctggaagcccaccatccccaccccctggcgttactacttccagtgggaccgtaccctgatcccctcccacaccggtacttccggcacccccaccaacatctaccacggcaccgaccccgacgacgtgcagttctacaccatcgagaactccgtgcccgtgcacctgctgcgtaccggtgacgagttcgctaccggaaccttcttcttcgactgcaagccctgccgtctgacccacacctggcagaccaaccgtgctctgggtctgcctcccttcctgaactccctgccccaggctgagggtggcaccaacttcggttacatcggtgtgcagcaggacaagcgtcgtggtgtgacccagatgggtaacaccaactacatcaccgaggctaccatcatgcgtcccgctgaggtcggctactccgctccctactactccttcgaggcttccacccagggccccttcaagacccccatcgctgctggtcgtggtggtgctcagaccgacgagaaccaggctgctgacggtgacccccgttacgctttcggtcgtcagcacggccaaaagaccaccaccaccggcgagacccccgagcgtttcacctacatcgctcaccaggacaccggtcgttaccccgagggcgactggattcagaacatcaacttcaacctgcccgtgaccgaggacaacgtgctgctgcccaccgaccccatcggtggcaagaccggtatcaactacactaacatcttcaacacctacggtcctctgaccgctctgaacaacgtgccccccgtgtaccccaacggccagatctgggacaaggagttcgacaccgacctgaagccccgtctgcacgtgaacgctcccttcgtgtgccagaacaactgccctggccagctgttcgtcaaggtggcccccaacctgaccaacgagtacgaccctgacgcttccgctaacatgtcccgtatcgtgacctactccgacttctggtggaagggcaagctggtgttcaaggccaagctgcgtgcttctcacacctggaaccccatccagcagatgtccatcaacgtggacaaccagttcaactacgtgccctccaacatcggtggaatgaagatcgtgtacgagaagtcccagctggctccccgtaagctgtac

SEQ ID NO: 6 - protein, 578 aa, Artificial Sequence
  Truncated CPV VP2 in pMEB073
MLKGGQPAVRNERATGSGNGSGGGGGGGSGGVGISTGTFNNQTEFKFLENGWVEITANSSRLVHLNMPESENYRRVVVNNLDKTAVNGNMALDDTHAQIVTPWSLVDANAWGVWFNPGDWQLIVNTMSELHLVSFEQEIFNVVLKTVSESATQPPTKVYNNDLTASLMVALDSNNTMPFTPAAMRSETLGFYPWKPTIPTPWRYYFQWDRTLIPSHTGTSGTPTNIYHGTDPDDVQFYTIENSVPVHLLRTGDEFATGTFFFDCKPCRLTHTWQTNRALGLPPFLNSLPQAEGGTNFGYIGVQQDKRRGVTQMGNTNYITEATIMRPAEVGYSAPYYSFEASTQGPFKTPIAAGRGGAQTDENQAADGDPRYAFGRQHGQKTTTTGETPERFTYIAHQDTGRYPEGDWIQNINFNLPVTEDNVLLPTDPIGGKTGINYTNIFNTYGPLTALNNVPPVYPNGQIWDKEFDTDLKPRLHVNAPFVCQNNCPGQLFVKVAPNLTNEYDPDASANMSRIVTYSDFWWKGKLVFKAKLRASHTWNPIQQMSINVDNQFNYVPSNIGGMKIVYEKSQLAPRKLY

SEQ ID NO: 7 - DNA, 1536 bp, Artificial Sequence
  pMEB073 codon-optimized nucleic acid sequence encoding CPV VP2 (SEQ ID NO:6)
atgcccgagagcgagaactaccggagagtggtggtgaacaacctggacaagaccgccgtgaacggcaatatggccctggatgacacccacgcccagatcgtgaccccctggagcctggtggacgccaacgcctggggagtgtggttcaaccctggcgactggcagctgatcgtgaacaccatgagcgagctgcacctggtgtccttcgagcaggagattttcaacgtggtgctgaaaaccgtgtccgagagcgccacccagccccccaccaaagtgtacaacaacgacctgaccgcctccctgatggtggccctggacagcaacaacaccatgcccttcacccctgccgccatgagaagcgagaccctgggcttctacccttggaagcccaccatccccaccccttggcggtactacttccagtgggacaggaccctgatccccagccacaccggcaccagcggcacccctaccaatatctaccacggcaccgaccctgatgacgtgcagttctacaccatcgagaacagcgtgcctgtgcacctgctgagaaccggcgacgagttcgccaccggcacattcttcttcgactgcaagccctgcagactgacccacacctggcagaccaacagagccctgggcctgcctcctttcctgaacagcctgccccaggccgagggcggcaccaacttcggctacatcggcgtgcagcaggacaagagaagaggcgtgacccagatgggcaacaccaactacatcaccgaggccaccatcatgagacccgccgaagtgggctacagcgccccctactacagcttcgaggccagcacccagggccccttcaagacccccatcgccgctggcagaggcggagcccagaccgacgagaaccaggccgccgacggcgaccccagatacgccttcggcagacagcacggccagaaaaccaccaccaccggcgagacccccgagagattcacctacatcgcccaccaggacaccggcagataccccgagggcgactggattcagaacatcaacttcaacctgcccgtgaccgaggataatgtgctgctgcccaccgaccccatcggcggcaagaccggcatcaactacaccaacatcttcaacacctacggccccctgaccgccctgaataacgtgccccccgtgtaccccaacggccagatttgggacaaggagttcgacaccgacctgaagcctaggctgcacgtgaatgcccccttcgtgtgtcagaacaactgccctggccagctgtttgtgaaagtggcccccaacctgaccaacgagtacgatcctgacgccagcgccaacatgagccggatcgtgacctacagcgacttctggtggaagggcaagctggtgttcaaggccaagctgagagccagccacacatggaaccccatccagcagatgagcatcaacgtggacaaccagttcaactacgtgcccagcaatatcggcggcatgaagatcgtgtacgagaagagccagctggcccccagaaagctgtac

SEQ ID NO: 8 - protein, 584 aa, Artificial Sequence
  GenBank: AHW47988.1
MSDGAVQPDGGQPAVRNERATGSGNGSGGGGGGGSGGVGISTGTFNNQTEFKFLENGWVEITANSSRLVHLNMPESENYKRVVVNNMDKTAVKGNMALDDTHVQIVTPWSLVDANAWGVWFNPGDWQLIVNTMSELHLVSFEREIFNVVLKTVSESATQPPTKVYNNDLTASLMVALDSNNTMPFTPAAMRSETLGFYPWKPTIPTPWRYYFQWDRTLIPSHTGTSGTPTNVYHGSDPDDVQFYTIENSVPVHLLRTGDEFATGTFFFDCKPCRLTHTWQTNRALGLPPFLNSLPQSEGITNFGDIGVQQDKRRGVTQMGNTDYITEATIMRPAEVGYSAPYYSFEASTQGPFKTPIAAGRGGAQTDENQAADGDPKYAFGRQHGQKTTTTGETPERFTYIAHQDTGRYPEGDWIQNINFNLPVTKDNVLLPTDPIGGKTGINYTNIFNTYGPLTALNNVPPVYPNGQIWDKEFDTDLKPRLHVNAPFVCQNNCPGQLFVKVAPNLTNEYDPDASANMSRIVTYSDFWWKGKLVFKAKLRASHTWNPIQQMSINVDNQFNYVPNNIGAMKIVYEKSQLAPRKLY

SEQ ID NO: 9 - protein, 584 aa, Artificial Sequence
  GenBank: AHW47989.1
MSDGAVQPDGGQPAVRNERATGSGNGSGGGGGGGSGGVGISTGTFNNQTEFKFLENGWVEITANSSRLVHLNMPESENYKRVVVNNMDKTAVKGNMALDDTHVQIVTPWSLVDANAWGVWFNPGDWQLIVNTMSELHLVSFEQEIFNVVLKTVSESATQPPTKVYNNDLTASLMVALDSNNTMPFTPAAMRSETLGFYPWKPTIPTPWRYYFQWDRTLIPSHTGTSGTPTNVYHGSDPDDVQFYTIENSVPVHLLRTGDEFATGTFFFDCKPCRLTHTWQTNRALGLPPFLNSLPQSEGITNFGDIGVQQDKRRGVTQMGNTDYITEATIMRPAEVGYSAPYYSFEASTQGPFKTPIAAGRGGAQTDENQAADGDPKYAFGRQHGQKTTTTGETPERFTYISHQDTGRYPEGDWIQNINFNLPVTKDNVLLPTDPIGGKTGINYTNIFNTYGPLTALNNVPPVYPNGQIWDKEFDTDLKPRLHVNAPFVCQNNCPGQLFVKVAPNLTNEYDPDASANMSRIVTYSDFWWKGKLVFKAKLRASHTWNPIQQMSINVDNQFNYVPNNIGAMKIVYEKSQLAPRKLY

SEQ ID NO: 10 - protein, 584 aa, Artificial Sequence
  GenBank: ADA61118.1
MSDGAVQPDGGQPAVRNERATGSGNGSGGGGGGGSGGGGISTGAFNNQTEFKFLENGWVEITANSSRLVHLNMPESENYRRVVVNNMDKTAVNGNMALDDIHAQIVTPWSLVDANAWGVWFNPGDWQLIVNTMSELHLVSFEQEIFNVVLKTVSESATQPPTKVYNNDLTASLMVALDSNNTMPFTPAAMRSETLGFYPWKPTIPTPWRYHFQWDRTLIPSHTGTSGTPTNIYHGTDPDDVQFYTIENSVPVHLLRTGDEFATGTFFFDCTPCRLTHTWQTNRALGLPPFLNSLPQSEGATNFGDIGVQQDKRRGVTQMGNTNYITEATIMRPAEVGYSAPYYSFEASTQGPFKTPIAAGRGGAQTDENQAADGEPRYAFGRQHGQKTTTTGETPERFTYIAHQDTGRYPEGDWIQNINFNLPVTNDNVLLPTDPIGGKTGINYTNIFNTYGPLTALNNVPPVYPNGQIWDKEFDTDLKPRLHVNAPFVCQNNCPGQLFVKVAPNLTNEYDPDASANMSRIVTYSDFWWKGKLVFKAKLRASHTWNPIQQMSINVDNQFNYVPSNIGGMKIVFEKSQLAPRKLY

SEQ ID NO: 11 - DNA, 11387 bp, Artificial Sequence
  pMEB072
aagctttactcgtaaagcgagttgaaggatcatatttagttgcgtttatgagataagattgaaagcacgtgtaaaatgtttcccgcgcgttggcacaactatttacaatgcggccaagttataaaagattctaatctgatatgttttaaaacacctttgcggcccgagttgtttgcgtacgtgactagcgaagaagatgtgtggaccgcagaacagatagtaaaacaaaaccctagtattggagcaataatcgatttaaccaacacgtctaaatattatgatggtgtgcattttttgcgggcgggcctgttatacaaaaaaattcaagtacctggccagactttgccgcctgaaagcatagttcaagaatttattgacacggtaaaagaatttacagaaaagtgtcccggcatgttggtgggcgtgcactgcacacacggtattaatcgcaccggttacatggtgtgcagatatttaatgcacaccctgggtattgcgccgcaggaagccatagatagattcgaaaaagccagaggtcacaaaattgaaagacaaaattacgttcaagatttattaatttaattaatattatttgcattctttaacaaatactttatcctattttcaaattgttgcgcttcttccagcgaaccaaaactatgcttcgcttgctccgtttagcttgtagccgatcagtggcgttgttccaatcgacggtaggattaggccggatattctccaccacaatgttggcaacgttgatgttacgtttatgcttttggttttccacgtacgtcttttggccggtaatagccgtaaacgtagtgccgtcgcgcgtcacgcacaacaccggatgtttgcgcttgtccgcggggtattgaaccgcgcgatccgacaaatccaccactttggcaactaaatcggtgacctgcgcgtcttttttctgcattatttcgtctttcttttgcatggtttcctggaagccggtgtacatgcggtttagatcagtcatgacgcgcgtgacctgcaaatctttggcctcgatctgcttgtccttgatggcaacgatgcgttcaataaactcttgttttttaacaagttcctcggttttttgcgccaccaccgcttgcagcgcgtttgtgtgctcggtgaatgtcgcaatcagcttagtcaccaactgtttgctctcctcctcccgttgtttgatcgcgggatcgtacttgccggtgcagagcacttgaggaattacttcttctaaaagccattcttgtaattctatggcgtaaggcaatttggacttcataatcagctgaatcacgccggatttagtaatgagcactgtatgcggctgcaaatacagcgggtcgccccttttcacgacgctgttagaggtagggcccccattttggatggtctgctcaaataacgatttgtatttattgtctacatgaacacgtatagctttatcacaaactgtatattttaaactgttagcgacgtccttggccacgaaccggacctgttggtcgcgctctagcacgtaccgcaggttgaacgtatcttctccaaatttaaattctccaattttaacgcgagccattttgatacacgtgtgtcgattttgcaacaactattgttttttaacgcaaactaaacttattgtggtaagcaataattaaatatgggggaacatgcgccgctacaacactcgtcgttatgaacgcagacggcgccggtctcggcgcaagcggctaaaacgtgttgcgcgttcaacgcggcaaacatcgcaaaagccaatagtacagttttgatttgcatattaacggcgattttttaaattatcttatttaataaatagttatgacgcctacaactccccgcccgcgttgactcgctgcacctcgagcagttcgttgacgccttcctccgtgtggccgaacacgtcgagcgggtggtcgatgaccagcggcgtgccgcacgcgacgcacaagtatctgtacaccgaatgatcgtcgggcgaaggcacgtcggcctccaagtggcaatattggcaaattcgaaaatatatacagttgggttgtttgcgcatatctatcgtggcgttgggcatgtacgtccgaacgttgatttgcatgcaagccgaaattaaatcattgcgattagtgcgattaaaacgttgtacatcctcgcttttaatcatgccgtcgattaaatcgcgcaatcgagtcaagtgatcaaagtgtggaataatgttttctttgtattcccgagtcaagcgcagcgcgtattttaacaaactagccatcttgtaagttagtttcatttaatgcaactttatccaataatatattatgtatcgcacgtcaagaattaacaatgcgcccgttgtcgcatctcaacacgactatgatagagatcaaataaagcgcgaattaaatagcttgcgacgcaacgtgcacgatctgtgcacgcgttccggcacgagctttgattgtaataagtttttacgaagcgatgacatgacccccgtagtgacaacgatcacgcccaaaagaactgccgactacaaaattaccgagtatgtcggtgacgttaaaactattaagccatccaatcgaccgttagtcgaatcaggaccgctggtgcgagaagccgcgaagtatggcgaatgcatcgtataacgtgtggagtccgctcattagagcgtcatgtttagacaagaaagctacatatttaattgatcccgatgattttattgataaattgaccctaactccatacacggtattctacaatggcggggttttggtcaaaatttccggactgcgattgtacatgctgttaacggctccgcccactattaatgaaattaaaaattccaattttaaaaaacgcagcaagagaaacatttgtatgaaagaatgcgtagaaggaaagaaaaatgtcgtcgacatgctgaacaacaagattaatatgcctccgtgtataaaaaaaatattgaacgatttgaaagaaaacaatgtaccgcgcggcggtatgtacaggaagaggtttatactaaactgttacattgcaaacgtggtttcgtgtgccaagtgtgaaaaccgatgtttaatcaaggctctgacgcatttctacaaccacgactccaagtgtgtgggtgaagtcatgcatcttttaatcaaatcccaagatgtgtataaaccaccaaactgccaaaaaatgaaaactgtcgacaagctctgtccgtttgctggcaactgcaagggtctcaatcctatttgtaattattgaataataaaacaattataaatgctaaatttgttttttattaacgatacaaaccaaacgcaacaagaacatttgtagtattatctataattgaaaacgcgtagttataatcgctgaggtaatatttaaaatcattttcaaatgattcacagttaatttgcgacaatataattttattttcacataaactagacgccttgtcgtcttcttcttcgtattccttctctttttcatttttctcctcataaaaattaacatagttattatcgtatccatatatgtatctatcgtatagagtaaattttttgttgtcataaatatatatgtcttttttaatggggtgtatagtaccgctgcgcatagtttttctgtaatttacaacagtgctattttctggtagttcttcggagtgtgttgctttaattattaaatttatataatcaatgaatttgggatcgtcggttttgtacaatatgttgccggcatagtacgcagcttcttctagttcaattacaccattttttagcagcaccggattaacataactttccaaaatgttgtacgaaccgttaaacaaaaacagttcacctcccttttctatactattgtctgcgagcagttgtttgttgttaaaaataacagccattgtaatgagacgcacaaactaatatcacaaactggaaatgtctatcaatatatagttgctgatatcatggagataattaaaatgataaccatctcgcaaataaataagtattttactgttttcgtaacagttttgtaataaaaaaacctataaatattccggattattcataccgtcccaccatcgggcgcggatccgccaccatgtccgacggtgctgtgcagcccgacggtggccagcccgctgtgcgtaacgagcgtgctaccggttccggtaacggttcaggcggaggtggaggtggtggttccggcggtgtgggcatctccaccggcaccttcaacaaccagaccgagttcaagttcctcgagaacggttgggtggagatcaccgctaactcctcccgtctggtgcacctgaacatgcccgagtccgagaactaccgtcgtgtggtggtgaacaacctggacaagaccgctgtgaacggtaacatggctctggacgacacccacgctcagatcgtgaccccctggtccctggtggacgctaacgcttggggcgtgtggttcaaccccggtgactggcagctgatcgtgaacaccatgtccgagctgcacctggtgtccttcgagcaagagatcttcaacgtcgtcctcaagaccgtgtccgagtccgctacccagccccccaccaaggtgtacaacaacgacctgaccgcttccctgatggtcgctctggactccaacaacaccatgcccttcacccccgctgctatgcgttccgagaccctgggcttctacccctggaagcccaccatccccaccccctggcgttactacttccagtgggaccgtaccctgatcccctcccacaccggtacttccggcacccccaccaacatctaccacggcaccgaccccgacgacgtgcagttctacaccatcgagaactccgtgcccgtgcacctgctgcgtaccggtgacgagttcgctaccggaaccttcttcttcgactgcaagccctgccgtctgacccacacctggcagaccaaccgtgctctgggtctgcctcccttcctgaactccctgccccaggctgagggtggcaccaacttcggttacatcggtgtgcagcaggacaagcgtcgtggtgtgacccagatgggtaacaccaactacatcaccgaggctaccatcatgcgtcccgctgaggtcggctactccgctccctactactccttcgaggcttccacccagggccccttcaagacccccatcgctgctggtcgtggtggtgctcagaccgacgagaaccaggctgctgacggtgacccccgttacgctttcggtcgtcagcacggccaaaagaccaccaccaccggcgagacccccgagcgtttcacctacatcgctcaccaggacaccggtcgttaccccgagggcgactggattcagaacatcaacttcaacctgcccgtgaccgaggacaacgtgctgctgcccaccgaccccatcggtggcaagaccggtatcaactacactaacatcttcaacacctacggtcctctgaccgctctgaacaacgtgccccccgtgtaccccaacggccagatctgggacaaggagttcgacaccgacctgaagccccgtctgcacgtgaacgctcccttcgtgtgccagaacaactgccctggccagctgttcgtcaaggtggcccccaacctgaccaacgagtacgaccctgacgcttccgctaacatgtcccgtatcgtgacctactccgacttctggtggaagggcaagctggtgttcaaggccaagctgcgtgcttctcacacctggaaccccatccagcagatgtccatcaacgtggacaaccagttcaactacgtgccctccaacatcggtggaatgaagatcgtgtacgagaagtcccagctggctccccgtaagctgtactaataatctagaattccggagcggccgctgcagatctgatcctttcctgggacccggcaagaaccaaaaactcactctcttcaaggaaatccgtaatgttaaacccgacacgatgaagcttgtcgttggatggaaaggaaaagagttctacagggaaacttggacccgcttcatggaagacagcttccccattgttaacgaccaagaagtgatggatgttttccttgttgtcaacatgcgtcccactagacccaaccgttgttacaaattcctggcccaacacgctctgcgttgcgaccccgactatgtacctcatgacgtgattaggatcgtcgagccttcatgggtgggcagcaacaacgagtaccgcatcagcctggctaagaagggcggcggctgcccaataatgaaccttcactctgagtacaccaactcgttcgaacagttcatcgatcgtgtcatctgggagaacttctacaagcccatcgtttacatcggtaccgactctgctgaagaggaggaaattctccttgaagtttccctggtgttcaaagtaaaggagtttgcaccagacgcacctctgttcactggtccggcgtattaaaacacgatacattgttattagtacatttattaagcgctagattctgtgcgttgttgatttacagacaattgttgtacgtattttaataattcattaaatttataatctttagggtggtatgttagagcgaaaatcaaatgattttcagcgtctttatatctgaatttaaatattaaatcctcaatagatttgtaaaataggtttcgattagtttcaaacaagggttgtttttccgaaccgatggctggactatctaatggattttcgctcaacgccacaaaacttgccaaatcttgtagcagcaatctagctttgtcgatattcgtttgtgttttgttttgtaataaaggttcgacgtcgttcaaaatattatgcgcttttgtatttctttcatcactgtcgttagtgtacaattgactcgacgtaaacacgttaaataaagcttggacatatttaacatcgggcgtgttagctttattaggccgattatcgtcgtcgtcccaaccctcgtcgttagaagttgcttccgaagacgattttgccatagccacacgacgcctattaattgtgtcggctaacacgtccgcgatcaaatttgtagttgagctttttggaattatttctgattgcgggcgtttttgggcgggtttcaatctaactgtgcccgattttaattcagacaacacgttagaaagcgatggtgcaggcggtggtaacatttcagacggcaaatctactaatggcggcggtggtggagctgatgataaatctaccatcggtggaggcgcaggcggggctggcggcggaggcggaggcggaggtggtggcggtgatgcagacggcggtttaggctcaaatgtctctttaggcaacacagtcggcacctcaactattgtactggtttcgggcgccgtttttggtttgaccggtctgagacgagtgcgatttttttcgtttctaatagcttccaacaattgttgtctgtcgtctaaaggtgcagcgggttgaggttccgtcggcattggtggagcgggcggcaattcagacatcgatggtggtggtggtggtggaggcgctggaatgttaggcacgggagaaggtggtggcggcggtgccgccggtataatttgttctggtttagtttgttcgcgcacgattgtgggcaccggcgcaggcgccgctggctgcacaacggaaggtcgtctgcttcgaggcagcgcttggggtggtggcaattcaatattataattggaatacaaatcgtaaaaatctgctataagcattgtaatttcgctatcgtttaccgtgccgatatttaacaaccgctcaatgtaagcaattgtattgtaaagagattgtctcaagctcgccgcacgccgataacaagccttttcatttttactacagcattgtagtggcgagacacttcgctgtcgtcgacgtacatgtatgctttgttgtcaaaaacgtcgttggcaagctttaaaatatttaaaagaacatctctgttcagcaccactgtgttgtcgtaaatgttgtttttgataatttgcgcttccgcagtatcgacacgttcaaaaaattgatgcgcatcaattttgttgttcctattattgaataaataagattgtacagattcatatctacgattcgtcatggccaccacaaatgctacgctgcaaacgctggtacaattttacgaaaactgcaaaaacgtcaaaactcggtataaaataatcaacgggcgctttggcaaaatatctattttatcgcacaagcccactagcaaattgtatttgcagaaaacaatttcggcgcacaattttaacgctgacgaaataaaagttcaccagttaatgagcgaccacccaaattttataaaaatctattttaatcacggttccatcaacaaccaagtgatcgtgatggactacattgactgtcccgatttatttgaaacactacaaattaaaggcgagctttcgtaccaacttgttagcaatattattagacagctgtgtgaagcgctcaacgatttgcacaagcacaatttcatacacaacgacataaaactcgaaaatgtcttatatttcgaagcacttgatcgcgtgtatgtttgcgattacggattgtgcaaacacgaaaactcacttagcgtgcacgacggcacgttggagtattttagtccggaaaaaattcgacacacaactatgcacgtttcgtttgactggtacgcggcgtgttaacatacaagttgctaacgtaatcatggtcatagctgtttcctgtgtgaaattgttatccgctcacaattccacacaacatacgagccggaagcataaagtgtaaagcctggggtgcctaatgagtgagctaactcacattaattgcgttgcgctcactgcccgctttccagtcgggaaacctgtcgtgccagctgcattaatgaatcggccaacgcgcggggagaggcggtttgcgtattgggcgctcttccgcttcctcgctcactgactcgctgcgctcggtcgttcggctgcggcgagcggtatcagctcactcaaaggcggtaatacggttatccacagaatcaggggataacgcaggaaagaacatgtgagcaaaaggccagcaaaaggccaggaaccgtaaaaaggccgcgttgctggcgtttttccataggctccgcccccctgacgagcatcacaaaaatcgacgctcaagtcagaggtggcgaaacccgacaggactataaagataccaggcgtttccccctggaagctccctcgtgcgctctcctgttccgaccctgccgcttaccggatacctgtccgcctttctcccttcgggaagcgtggcgctttctcatagctcacgctgtaggtatctcagttcggtgtaggtcgttcgctccaagctgggctgtgtgcacgaaccccccgttcagcccgaccgctgcgccttatccggtaactatcgtcttgagtccaacccggtaagacacgacttatcgccactggcagcagccactggtaacaggattagcagagcgaggtatgtaggcggtgctacagagttcttgaagtggtggcctaactacggctacactagaaggacagtatttggtatctgcgctctgctgaagccagttaccttcggaaaaagagttggtagctcttgatccggcaaacaaaccaccgctggtagcggtggtttttttgtttgcaagcagcagattacgcgcagaaaaaaaggatctcaagaagatcctttgatcttttctacggggtctgacgctcagtggaacgaaaactcacgttaagggattttggtcatgagattatcaaaaaggatcttcacctagatccttttaaattaaaaatgaagttttaaatcaatctaaagtatatatgagtaaacttggtctgacagttaccaatgcttaatcagtgaggcacctatctcagcgatctgtctatttcgttcatccatagttgcctgactccccgtcgtgtagataactacgatacgggagggcttaccatctggccccagtgctgcaatgataccgcgagacccacgctcaccggctccagatttatcagcaataaaccagccagccggaagggccgagcgcagaagtggtcctgcaactttatccgcctccatccagtctattaattgttgccgggaagctagagtaagtagttcgccagttaatagtttgcgcaacgttgttgccattgctacaggcatcgtggtgtcacgctcgtcgtttggtatggcttcattcagctccggttcccaacgatcaaggcgagttacatgatcccccatgttgtgcaaaaaagcggttagctccttcggtcctccgatcgttgtcagaagtaagttggccgcagtgttatcactcatggttatggcagcactgcataattctcttactgtcatgccatccgtaagatgcttttctgtgactggtgagtactcaaccaagtcattctgagaatagtgtatgcggcgaccgagttgctcttgcccggcgtcaatacgggataataccgcgccacatagcagaactttaaaagtgctcatcattggaaaacgttcttcggggcgaaaactctcaaggatcttaccgctgttgagatccagttcgatgtaacccactcgtgcacccaactgatcttcagcatcttttactttcaccagcgtttctgggtgagcaaaaacaggaaggcaaaatgccgcaaaaaagggaataagggcgacacggaaatgttgaatactcatactcttcctttttcaatattattgaagcatttatcagggttattgtctcatgagcggatacatatttgaatgtatttagaaaaataaacaaataggggttccgcgcacatttccccgaaaagtgccacctgacgtctaagaaaccattattatcatgacattaacctataaaaataggcgtatcacgaggccctttcgtctcgcgcgtttcggtgatgacggtgaaaacctctgacacatgcagctcccggagacggtcacagcttgtctgtaagcggatgccgggagcagacaagcccgtcagggcgcgtcagcgggtgttggcgggtgtcggggctggcttaactatgcggcatcagagcagattgtactgagagtgcaccatatgcggtgtgaaataccgcacagatgcgtaaggagaaaataccgcatcaggcgccattcgccattcaggctgcgcaactgttgggaagggcgatcggtgcgggcctcttcgctattacgccagctggcgaaagggggatgtgctgcaaggcgattaagttgggtaacgccagggttttcccagtcacgacgttgtaaaacgacggccagtgcc

SEQ ID NO: 12 - DNA, 11385 bp, Artificial Sequence
  pMEB073
ctagaattccggagcggccgctgcagatctgatcctttcctgggacccggcaagaaccaaaaactcactctcttcaaggaaatccgtaatgttaaacccgacacgatgaagcttgtcgttggatggaaaggaaaagagttctacagggaaacttggacccgcttcatggaagacagcttccccattgttaacgaccaagaagtgatggatgttttccttgttgtcaacatgcgtcccactagacccaaccgttgttacaaattcctggcccaacacgctctgcgttgcgaccccgactatgtacctcatgacgtgattaggatcgtcgagccttcatgggtgggcagcaacaacgagtaccgcatcagcctggctaagaagggcggcggctgcccaataatgaaccttcactctgagtacaccaactcgttcgaacagttcatcgatcgtgtcatctgggagaacttctacaagcccatcgtttacatcggtaccgactctgctgaagaggaggaaattctccttgaagtttccctggtgttcaaagtaaaggagtttgcaccagacgcacctctgttcactggtccggcgtattaaaacacgatacattgttattagtacatttattaagcgctagattctgtgcgttgttgatttacagacaattgttgtacgtattttaataattcattaaatttataatctttagggtggtatgttagagcgaaaatcaaatgattttcagcgtctttatatctgaatttaaatattaaatcctcaatagatttgtaaaataggtttcgattagtttcaaacaagggttgtttttccgaaccgatggctggactatctaatggattttcgctcaacgccacaaaacttgccaaatcttgtagcagcaatctagctttgtcgatattcgtttgtgttttgttttgtaataaaggttcgacgtcgttcaaaatattatgcgcttttgtatttctttcatcactgtcgttagtgtacaattgactcgacgtaaacacgttaaataaagcttggacatatttaacatcgggcgtgttagctttattaggccgattatcgtcgtcgtcccaaccctcgtcgttagaagttgcttccgaagacgattttgccatagccacacgacgcctattaattgtgtcggctaacacgtccgcgatcaaatttgtagttgagctttttggaattatttctgattgcgggcgtttttgggcgggtttcaatctaactgtgcccgattttaattcagacaacacgttagaaagcgatggtgcaggcggtggtaacatttcagacggcaaatctactaatggcggcggtggtggagctgatgataaatctaccatcggtggaggcgcaggcggggctggcggcggaggcggaggcggaggtggtggcggtgatgcagacggcggtttaggctcaaatgtctctttaggcaacacagtcggcacctcaactattgtactggtttcgggcgccgtttttggtttgaccggtctgagacgagtgcgatttttttcgtttctaatagcttccaacaattgttgtctgtcgtctaaaggtgcagcgggttgaggttccgtcggcattggtggagcgggcggcaattcagacatcgatggtggtggtggtggtggaggcgctggaatgttaggcacgggagaaggtggtggcggcggtgccgccggtataatttgttctggtttagtttgttcgcgcacgattgtgggcaccggcgcaggcgccgctggctgcacaacggaaggtcgtctgcttcgaggcagcgcttggggtggtggcaattcaatattataattggaatacaaatcgtaaaaatctgctataagcattgtaatttcgctatcgtttaccgtgccgatatttaacaaccgctcaatgtaagcaattgtattgtaaagagattgtctcaagctccgcacgccgataacaagccttttcatttttactacagcattgtagtggcgagacacttcgctgtcgtcgacgtacatgtatgctttgttgtcaaaaacgtcgttggcaagctttaaaatatttaaaagaacatctctgttcagcaccactgtgttgtcgtaaatgttgtttttgataatttgcgcttccgcagtatcgacacgttcaaaaaattgatgcgcatcaattttgttgttcctattattgaataaataagattgtacagattcatatctacgattcgtcatggccaccacaaatgctacgctgcaaacgctggtacaattttacgaaaactgcaaaaacgtcaaaactcggtataaaataatcaacgggcgctttggcaaaatatctattttatcgcacaagcccactagcaaattgtatttgcagaaaacaatttcggcgcacaattttaacgctgacgaaataaaagttcaccagttaatgagcgaccacccaaattttataaaaatctattttaatcacggttccatcaacaaccaagtgatcgtgatggactacattgactgtcccgatttatttgaaacactacaaattaaaggcgagctttcgtaccaacttgttagcaatattattagacagctgtgtgaagcgctcaacgatttgcacaagcacaatttcatacacaacgacataaaactcgaaaatgtcttatatttcgaagcacttgatcgcgtgtatgtttgcgattacggattgtgcaaacacgaaaactcacttagcgtgcacgacggcacgttggagtattttagtccggaaaaaattcgacacacaactatgcacgtttcgtttgactggtacgcggcgtgttaacatacaagttgctaaccggcggttcgtaatcatggtcatagctgtttcctgtgtgaaattgttatccgctcacaattccacacaacatacgagccggaagcataaagtgtaaagcctggggtgcctaatgagtgagctaactcacattaattgcgttgcgctcactgcccgctttccagtcgggaaacctgtcgtgccagctgcattaatgaatcggccaacgcgcggggagaggcggtttgcgtattgggcgctcttccgcttcctcgctcactgactcgctgcgctcggtcgttcggctgcggcgagcggtatcagctcactcaaaggcggtaatacggttatccacagaatcaggggataacgcaggaaagaacatgtgagcaaaaggccagcaaaaggccaggaaccgtaaaaaggccgcgttgctggcgtttttccataggctccgcccccctgacgagcatcacaaaaatcgacgctcaagtcagaggtggcgaaacccgacaggactataaagataccaggcgtttccccctggaagctccctcgtgcgctctcctgttccgaccctgccgcttaccggatacctgtccgcctttctcccttcgggaagcgtggcgctttctcatagctcacgctgtaggtatctcagttcggtgtaggtcgttcgctccaagctgggctgtgtgcacgaaccccccgttcagcccgaccgctgcgccttatccggtaactatcgtcttgagtccaacccggtaagacacgacttatcgccactggcagcagccactggtaacaggattagcagagcgaggtatgtaggcggtgctacagagttcttgaagtggtggcctaactacggctacactagaaggacagtatttggtatctgcgctctgctgaagccagttaccttcggaaaaagagttggtagctcttgatccggcaaacaaaccaccgctggtagcggtggtttttttgtttgcaagcagcagattacgcgcagaaaaaaaggatctcaagaagatcctttgatcttttctacggggtctgacgctcagtggaacgaaaactcacgttaagggattttggtcatgagattatcaaaaaggatcttcacctagatccttttaaattaaaaatgaagttttaaatcaatctaaagtatatatgagtaaacttggtctgacagttaccaatgcttaatcagtgaggcacctatctcagcgatctgtctatttcgttcatccatagttgcctgactccccgtcgtgtagataactacgatacgggagggcttaccatctggccccagtgctgcaatgataccgcgagacccacgctcaccggctccagatttatcagcaataaaccagccagccggaagggccgagcgcagaagtggtcctgcaactttatccgcctccatccagtctattaattgttgccgggaagctagagtaagtagttcgccagttaatagtttgcgcaacgttgttgccattgctacaggcatcgtggtgtcacgctcgtcgtttggtatggcttcattcagctccggttcccaacgatcaaggcgagttacatgatcccccatgttgtgcaaaaaagcggttagctccttcggtcctccgatcgttgtcagaagtaagttggccgcagtgttatcactcatggttatggcagcactgcataattctcttactgtcatgccatccgtaagatgcttttctgtgactggtgagtactcaaccaagtcattctgagaatagtgtatgcggcgaccgagttgctcttgcccggcgtcaatacgggataataccgcgccacatagcagaactttaaaagtgctcatcattggaaaacgttcttcggggcgaaaactctcaaggatcttaccgctgttgagatccagttcgatgtaacccactcgtgcacccaactgatcttcagcatcttttactttcaccagcgtttctgggtgagcaaaaacaggaaggcaaaatgccgcaaaaaagggaataagggcgacacggaaatgttgaatactcatactcttcctttttcaatattattgaagcatttatcagggttattgtctcatgagcggatacatatttgaatgtatttagaaaaataaacaaataggggttccgcgcacatttccccgaaaagtgccacctgacgtctaagaaaccattattatcatgacattaacctataaaaataggcgtatcacgaggccctttcgtctcgcgcgtttcggtgatgacggtgaaaacctctgacacatgcagctcccggagacggtcacagcttgtctgtaagcggatgccgggagcagacaagcccgtcagggcgcgtcagcgggtgttggcgggtgtcggggctggcttaactatgcggcatcagagcagattgtactgagagtgcaccatatgcggtgtgaaataccgcacagatgcgtaaggagaaaataccgcatcaggcgccattcgccattcaggctgcgcaactgttgggaagggcgatcggtgcgggcctcttcgctattacgccagctggcgaaagggggatgtgctgcaaggcgattaagttgggtaacgccagggttttcccagtcacgacgttgtaaaacgacggccagtgccaagctttactcgtaaagcgagttgaaggatcatatttagttgcgtttatgagataagattgaaagcacgtgtaaaatgtttcccgcgcgttggcacaactatttacaatgcggccaagttataaaagattctaatctgatatgttttaaaacacctttgcggcccgagttgtttgcgtacgtgactagcgaagaagatgtgtggaccgcagaacagatagtaaaacaaaaccctagtattggagcaataatcgatttaaccaacacgtctaaatattatgatggtgtgcattttttgcgggcgggcctgttatacaaaaaaattcaagtacctggccagactttgccgcctgaaagcatagttcaagaatttattgacacggtaaaagaatttacagaaaagtgtcccggcatgttggtgggcgtgcactgcacacacggtattaatcgcaccggttacatggtgtgcagatatttaatgcacaccctgggtattgcgccgcaggaagccatagatagattcgaaaaagccagaggtcacaaaattgaaagacaaaattacgttcaagatttattaatttaattaatattatttgcattctttaacaaatactttatcctattttcaaattgttgcgcttcttccagcgaaccaaaactatgcttcgcttgctccgtttagcttgtagccgatcagtggcgttgttccaatcgacggtaggattaggccggatattctccaccacaatgttggcaacgttgatgttacgtttatgcttttggttttccacgtacgtcttttggccggtaatagccgtaaacgtagtgccgtcgcgcgtcacgcacaacaccggatgtttgcgcttgtccgcggggtattgaaccgcgcgatccgacaaatccaccactttggcaactaaatcggtgacctgcgcgtcttttttctgcattatttcgtctttcttttgcatggtttcctggaagccggtgtacatgcggtttagatcagtcatgacgcgcgtgacctgcaaatctttggcctcgatctgcttgtccttgatggcaacgatgcgttcaataaactcttgttttttaacaagttcctcggttttttgcgccaccaccgcttgcagcgcgtttgtgtgctcggtgaatgtcgcaatcagcttagtcaccaactgtttgctctcctcctcccgttgtttgatcgcgggatcgtacttgccggtgcagagcacttgaggaattacttcttctaaaagccattcttgtaattctatggcgtaaggcaatttggacttcataatcagctgaatcacgccggatttagtaatgagcactgtatgcggctgcaaatacagcgggtcgccccttttcacgacgctgttagaggtagggcccccattttggatggtctgctcaaataacgatttgtatttattgtctacatgaacacgtatagctttatcacaaactgtatattttaaactgttagcgacgtccttggccacgaaccggacctgttggtcgcgctctagcacgtaccgcaggttgaacgtatcttctccaaatttaaattctccaattttaacgcgagccattttgatacacgtgtgtcgattttgcaacaactattgttttttaacgcaaactaaacttattgtggtaagcaataattaaatatgggggaacatgcgccgctacaacactcgtcgttatgaacgcagacggcgccggtctcggcgcaagcggctaaaacgtgttgcgcgttcaacgcggcaaacatcgcaaaagccaatagtacagttttgatttgcatattaacggcgattttttaaattatcttatttaataaatagttatgacgcctacaactccccgcccgcgttgactcgctgcacctcgagcagttcgttgacgccttcctccgtgtggccgaacacgtcgagcgggtggtcgatgaccagcggcgtgccgcacgcgacgcacaagtatctgtacaccgaatgatcgtcgggcgaaggcacgtcggcctccaagtggcaatattggcaaattcgaaaatatatacagttgggttgtttgcgcatatctatcgtggcgttgggcatgtacgtccgaacgttgatttgcatgcaagccgaaattaaatcattgcgattagtgcgattaaaacgttgtacatcctcgcttttaatcatgccgtcgattaaatcgcgcaatcgagtcaagtgatcaaagtgtggaataatgttttctttgtattcccgagtcaagcgcagcgcgtattttaacaaactagccatcttgtaagttagtttcatttaatgcaactttatccaataatatattatgtatcgcacgtcaagaattaacaatgcgcccgttgtcgcatctcaacacgactatgatagagatcaaataaagcgcgaattaaatagcttgcgacgcaacgtgcacgatctgtgcacgcgttccggcacgagctttgattgtaataagtttttacgaagcgatgacatgacccccgtagtgacaacgatcacgcccaaaagaactgccgactacaaaattaccgagtatgtcggtgacgttaaaactattaagccatccaatcgaccgttagtcgaatcaggaccgctggtgcgagaagccgcgaagtatggcgaatgcatcgtataacgtgtggagtccgctcattagagcgtcatgtttagacaagaaagctacatatttaattgatcccgatgattttattgataaattgaccctaactccatacacggtattctacaatggcggggttttggtcaaaatttccggactgcgattgtacatgctgttaacggctccgcccactattaatgaaattaaaaattccaattttaaaaaacgcagcaagagaaacatttgtatgaaagaatgcgtagaaggaaagaaaaatgtcgtcgacatgctgaacaacaagattaatatgcctccgtgtataaaaaaaatattgaacgatttgaaagaaaacaatgtaccgcgcggcggtatgtacaggaagaggtttatactaaactgttacattgcaaacgtggtttcgtgtgccaagtgtgaaaaccgatgtttaatcaaggctctgacgcatttctacaaccacgactccaagtgtgtgggtgaagtcatgcatcttttaatcaaatcccaagatgtgtataaaccaccaaactgccaaaaaatgaaaactgtcgacaagctctgtccgtttgctggcaactgcaagggtctcaatcctatttgtaattattgaataataaaacaattataaatgctaaatttgttttttattaacgatacaaaccaaacgcaacaagaacatttgtagtattatctataattgaaaacgcgtagttataatcgctgaggtaatatttaaaatcattttcaaatgattcacagttaatttgcgacaatataattttattttcacataaactagacgccttgtcgtcttcttcttcgtattccttctctttttcatttttctcctcataaaaattaacatagttattatcgtatccatatatgtatctatcgtatagagtaaattttttgttgtcataaatatatatgtcttttttaatggggtgtatagtaccgctgcgcatagtttttctgtaatttacaacagtgctattttctggtagttcttcggagtgtgttgctttaattattaaatttatataatcaatgaatttgggatcgtcggttttgtacaatatgttgccggcatagtacgcagcttcttctagttcaattacaccattttttagcagcaccggattaacataactttccaaaatgttgtacgaaccgttaaacaaaaacagttcacctcccttttctatactattgtctgcgagcagttgtttgttgttaaaaataacagccattgtaatgagacgcacaaactaatatcacaaactggaaatgtctatcaatatatagttgctgatatcatggagataattaaaatgataaccatctcgcaaataaataagtattttactgttttcgtaacagttttgtaataaaaaaacctataaatattccggattattcataccgtcccaccatcgggcgcggatcccgggtcgacgccaccatgctgaagggcggccagcctgctgtgagaaacgagagagccaccggcagcggcaatggcagcggcggagggggcggaggaggatctggcggagtgggcatcagcaccggcaccttcaacaaccagaccgagttcaagttcctggagaacggctgggtggagatcaccgccaacagcagcagactggtgcacctgaacatgcccgagagcgagaactaccggagagtggtggtgaacaacctggacaagaccgccgtgaacggcaatatggccctggatgacacccacgcccagatcgtgaccccctggagcctggtggacgccaacgcctggggagtgtggttcaaccctggcgactggcagctgatcgtgaacaccatgagcgagctgcacctggtgtccttcgagcaggagattttcaacgtggtgctgaaaaccgtgtccgagagcgccacccagccccccaccaaagtgtacaacaacgacctgaccgcctccctgatggtggccctggacagcaacaacaccatgcccttcacccctgccgccatgagaagcgagaccctgggcttctacccttggaagcccaccatccccaccccttggcggtactacttccagtgggacaggaccctgatccccagccacaccggcaccagcggcacccctaccaatatctaccacggcaccgaccctgatgacgtgcagttctacaccatcgagaacagcgtgcctgtgcacctgctgagaaccggcgacgagttcgccaccggcacattcttcttcgactgcaagccctgcagactgacccacacctggcagaccaacagagccctgggcctgcctcctttcctgaacagcctgccccaggccgagggcggcaccaacttcggctacatcggcgtgcagcaggacaagagaagaggcgtgacccagatgggcaacaccaactacatcaccgaggccaccatcatgagacccgccgaagtgggctacagcgccccctactacagcttcgaggccagcacccagggccccttcaagacccccatcgccgctggcagaggcggagcccagaccgacgagaaccaggccgccgacggcgaccccagatacgccttcggcagacagcacggccagaaaaccaccaccaccggcgagacccccgagagattcacctacatcgcccaccaggacaccggcagataccccgagggcgactggattcagaacatcaacttcaacctgcccgtgaccgaggataatgtgctgctgcccaccgaccccatcggcggcaagaccggcatcaactacaccaacatcttcaacacctacggccccctgaccgccctgaataacgtgccccccgtgtaccccaacggccagatttgggacaaggagttcgacaccgacctgaagcctaggctgcacgtgaatgcccccttcgtgtgtcagaacaactgccctggccagctgtttgtgaaagtggcccccaacctgaccaacgagtacgatcctgacgccagcgccaacatgagccggatcgtgacctacagcgacttctggtggaagggcaagctggtgttcaaggccaagctgagagccagccacacatggaaccccatccagcagatgagcatcaacgtggacaaccagttcaactacgtgcccagcaatatcggcggcatgaagatcgtgtacgagaagagccagctggcccccagaaagctgtactgataat